European Patent Application EP 4 495 226 A1, published January 22, 2025. Title: MICROORGANISM WITH ENHANCED ACTIVITY OF ASPARTATE 1-DECARBOXYLASE FROM TRIBOLIUM CASTANEUM AND USES THEREOF. Applicant: CJ CheilJedang Corporation. The sequence listing filed with the application follows.

SEQUENCE LISTING (38 sequences)

SEQ ID NO: 1 - DNA, 36 bp, synthetic construct
  misc_feature 1..36: note = synthetic_primer
  source 1..36: mol_type = other DNA
tagatcgaaaggtgcacaaagatgattcgcacgatg

SEQ ID NO: 2 - DNA, 36 bp, synthetic construct
  misc_feature 1..36: note = synthetic_primer
  source 1..36: mol_type = other DNA
ccgctctagaactagtggatctcaagcaacctgtac

SEQ ID NO: 3 - DNA, 36 bp, synthetic construct
  misc_feature 1..36: note = synthetic_primer
  source 1..36: mol_type = other DNA
tagatcgaaaggtgcacaaagatgaagctgaccatc

SEQ ID NO: 4 - DNA, 36 bp, synthetic construct
  misc_feature 1..36: note = synthetic_primer
  source 1..36: mol_type = other DNA
ccgctctagaactagtggatcttaacacttctccca

SEQ ID NO: 5 - DNA, 36 bp, synthetic construct; identical to SEQ ID NO: 1
  misc_feature 1..36: note = synthetic_primer
  source 1..36: mol_type = other DNA

SEQ ID NO: 6 - DNA, 36 bp, synthetic construct; identical to SEQ ID NO: 2
  misc_feature 1..36: note = synthetic_primer
  source 1..36: mol_type = other DNA

SEQ ID NO: 7 - DNA, 37 bp, synthetic construct
  misc_feature 1..37: note = synthetic_primer
  source 1..37: mol_type = other DNA
tagatcgaaaggtgcacaaagatgatacgtactatgc

SEQ ID NO: 8 - DNA, 36 bp, synthetic construct
  misc_feature 1..36: note = synthetic_primer
  source 1..36: mol_type = other DNA
ccgctctagaactagtggatctcaggcaacctgtac

SEQ ID NO: 9 - DNA, 36 bp, synthetic construct
  misc_feature 1..36: note = synthetic_primer
  source 1..36: mol_type = other DNA
tagatcgaaaggtgcacaaagatgaaactcactatc

SEQ ID NO: 10 - DNA, 36 bp, synthetic construct
  misc_feature 1..36: note = synthetic_primer
  source 1..36: mol_type = other DNA
ccgctctagaactagtggatctcatttctgccagat

SEQ ID NO: 11 - DNA, 36 bp, synthetic construct
  misc_feature 1..36: note = synthetic_primer
  source 1..36: mol_type = other DNA
tagatcgaaaggtgcacaaagatgctgcgcaccatc

SEQ ID NO: 12 - DNA, 37 bp, synthetic construct
  misc_feature 1..37: note = synthetic_primer
  source 1..37: mol_type = other DNA
ccgctctagaactagtggatcctaaatgcttctcgac

SEQ ID NO: 13 - DNA, 36 bp, synthetic construct
  misc_feature 1..36: note = synthetic_primer
  source 1..36: mol_type = other DNA
tagatcgaaaggtgcacaaagatgcacgccataatg

SEQ ID NO: 14 - DNA, 36 bp, synthetic construct
  misc_feature 1..36: note = synthetic_primer
  source 1..36: mol_type = other DNA
ccgctctagaactagtggatctcaggcgacctgtat

SEQ ID NO: 15 - DNA, 36 bp, synthetic construct
  misc_feature 1..36: note = synthetic_primer
  source 1..36: mol_type = other DNA
tagatcgaaaggtgcacaaagatgccggcaaccgga

SEQ ID NO: 16 - DNA, 37 bp, synthetic construct
  misc_feature 1..37: note = synthetic_primer
  source 1..37: mol_type = other DNA
ccgctctagaactagtggatctggttcagatttgtaa

SEQ ID NO: 17 - DNA, 41 bp, synthetic construct
  misc_feature 1..41: note = synthetic_primer
  source 1..41: mol_type = other DNA
cttgatatcgaattcctgcattcagggtagttgactaaaga

SEQ ID NO: 18 - DNA, 17 bp, synthetic construct
  misc_feature 1..17: note = synthetic_primer
  source 1..17: mol_type = other DNA
ctttgtgcacctttcga

SEQ ID NO: 19 - DNA, 35 bp, synthetic construct
  misc_feature 1..35: note = synthetic_primer
  source 1..35: mol_type = other DNA
attcgagctcggtacccggcctcacggatcgtggt

SEQ ID NO: 20 - DNA, 33 bp, synthetic construct
  misc_feature 1..33: note = synthetic_primer
  source 1..33: mol_type = other DNA
agctaaaacgcccggggtcctgtggtgtcctta

SEQ ID NO: 21 - DNA, 35 bp, synthetic construct
  misc_feature 1..35: note = synthetic_primer
  source 1..35: mol_type = other DNA
aggacaccacaggaccccgggcgttttagctcgcc

SEQ ID NO: 22 - DNA, 35 bp, synthetic construct
  misc_feature 1..35: note = synthetic_primer
  source 1..35: mol_type = other DNA
tcgactctagaggatcccctctcatcggcgtgctg

SEQ ID NO: 23 - DNA, 34 bp, synthetic construct
  misc_feature 1..34: note = synthetic_primer
  source 1..34: mol_type = other DNA
aggacaccacaggaccccttcagggtagttgact

SEQ ID NO: 24 - DNA, 34 bp, synthetic construct
  misc_feature 1..34: note = synthetic_primer
  source 1..34: mol_type = other DNA
tggcgagctaaaacgcccttacaaatctgaacca

SEQ ID NO: 25 - DNA, 16 bp, synthetic construct
  misc_feature 1..16: note = synthetic_primer
  source 1..16: mol_type = other DNA
tctagatcagcgattg

SEQ ID NO: 26 - DNA, 16 bp, synthetic construct
  misc_feature 1..16: note = synthetic_primer
  source 1..16: mol_type = other DNA
atcgcgcactaaccga

SEQ ID NO: 27 - protein, 540 aa, synthetic construct
  REGION 1..540: note = synthetic_PanD from Tribolium castaneum (wild type)
MPATGEDQDLVQDLIEEPATFSDAVLSSDEELFHQKCPKPAPIYSPVSKPVSFESLPNRRLHEEFLRSSVDVLLQEAVFEGTNRKNRVLQWREPEELRRLMDFGVRSAPSTHEELLEVLKKVVTYSVKTGHPYFVNQLFSAVDPYGLVAQWATDALNPSVYTYEVSPVFVLMEEVVLREMRAIVGFEGGKGDGIFCPGGSIANGYAISCARYRFMPDIKKKGLHSLPRLVLFTSEDAHYSIKKLASFQGIGTDNVYLIRTDARGRMDVSHLVEEIERSLREGAAPFMVSATAGTTVIGAFDPIEKIADVCQKYKLWLHVDAAWGGGALVSAKHRHLLKGIERADSVTWNPHKLLTAPQQCSTLLLRHEGVLAEAHSTNAAYLFQKDKFYDTKYDTGDKHIQCGRRADVLKFWFMWKAKGTSGLEKHVDKVFENARFFTDCIKNREGFEMVIAEPEYTNICFWYVPKSLRGRKDEADYKDKLHKVAPRIKERMMKEGSMMVTYQAQKGHPNFFRIVFQNSGLDKADMVHLVEEIERLGSDL

SEQ ID NO: 28 - DNA, 40 bp, synthetic construct
  misc_feature 1..40: note = synthetic_primer
  source 1..40: mol_type = other DNA
tgaattcgagctcggtacccgaaatagcgcttgatgaatc

SEQ ID NO: 29 - DNA, 40 bp, synthetic construct
  misc_feature 1..40: note = synthetic_primer
  source 1..40: mol_type = other DNA
ggttgctacctgcacccggggggcatgagtatagatgtga

SEQ ID NO: 30 - DNA, 40 bp, synthetic construct
  misc_feature 1..40: note = synthetic_primer
  source 1..40: mol_type = other DNA
ctatactcatgccccccgggtgcaggtagcaaccacaaag

SEQ ID NO: 31 - DNA, 40 bp, synthetic construct
  misc_feature 1..40: note = synthetic_primer
  source 1..40: mol_type = other DNA
gtcgactctagaggatcccctatgtggcgttgggtgcagc

SEQ ID NO: 32 - DNA, 37 bp, synthetic construct
  misc_feature 1..37: note = synthetic_primer
  source 1..37: mol_type = other DNA
tagatcgaaaggtgcacaaagatgaaaccgaccacca

SEQ ID NO: 33 - DNA, 41 bp, synthetic construct
  misc_feature 1..41: note = synthetic_primer
  source 1..41: mol_type = other DNA
ccgctctagaactagtggatcttaatggaaactgtgttctt

SEQ ID NO: 34 - DNA, 35 bp, synthetic construct
  misc_feature 1..35: note = synthetic_primer
  source 1..35: mol_type = other DNA
catctatactcatgccccccttcagggtagttgac

SEQ ID NO: 35 - DNA, 35 bp, synthetic construct
  misc_feature 1..35: note = synthetic_primer
  source 1..35: mol_type = other DNA
ggtggtcggtttcatctttgtgcacctttcgatct

SEQ ID NO: 36 - DNA, 20 bp, synthetic construct
  misc_feature 1..20: note = synthetic_primer
  source 1..20: mol_type = other DNA
cccacccggtgtcattcgac

SEQ ID NO: 37 - DNA, 19 bp, synthetic construct
  misc_feature 1..19: note = synthetic_primer
  source 1..19: mol_type = other DNA
gcgcatccagctcatcggt

SEQ ID NO: 38 - DNA, 1623 bp, synthetic construct
  misc_feature 1..1623: note = synthetic_gene coding PanD from Tribolium castaneum (wild type)
  source 1..1623: mol_type = other DNA
atgccggcaaccggagaggaccaagacttggttcaggacttgatcgaggaacctgccactttcagcgacgctgtgttgtcctccgacgaggaactgtttcaccagaaatgcccgaagccggcaccaatttactcgccagtgtcaaaacccgtttcattcgagagcctgcccaatcgccgccttcatgaagaatttctccgctcatcggttgatgtactcctgcaggaggccgttttcgagggaactaatcggaagaatcgggtgcttcagtggcgtgagccagaggaattgcggcgtctcatggattttggcgttcggtctgctccttcaacccacgaagaactgctggaagttcttaaaaaagtagtcacgtacagcgtcaagaccggccacccctactttgtaaatcaactcttcagcgctgtcgacccctatggcctggtcgcgcaatgggctaccgatgccttgaatccctcagtgtacacgtacgaagttagcccggtcttcgtccttatggaggaagtcgtcctgcgtgaaatgcgtgcgattgtcggctttgagggaggcaagggagacggaattttctgtccaggtggctctatcgccaacggttacgcaatttcgtgtgcacggtatcgtttcatgccggatattaagaaaaaaggactgcactcacttccacggctggtactcttcacctcggaagacgctcactactcgatcaaaaaactggcatccttccagggcatcggcaccgataacgtttaccttatccgtactgatgcacggggccggatggatgtttctcacctggtggaggaaattgagcgctcgttgcgtgagggtgccgccccgttcatggtatccgccaccgcaggtacgacggtgatcggagcttttgaccctatcgaaaagatcgccgatgtctgccagaaatacaaattgtggctccacgttgacgctgcctggggtggaggagccttggtctcggctaagcatcgccatctgctcaaaggcatcgagcgggctgattctgttacgtggaatcctcataaactgcttaccgcaccccaacagtgcagcactttgcttcttcgccatgaaggcgtactggcggaagcacatagcaccaatgctgcttacctgttccagaaggacaagttttacgacaccaaatacgacaccggcgataaacacatccaatgtggtcggcgtgccgacgtgttgaaattctggttcatgtggaaggctaaaggcacctccggcttggaaaaacacgttgataaggtatttgaaaacgctcggttctttaccgactgtattaaaaaccgtgagggattcgagatggtaattgctgagccagagtatacgaacatctgtttctggtacgtaccaaaatccctgcggggccggaaggatgaagctgattataaagacaaattgcataaagtcgctccacgtatcaaggaacgcatgatgaaagagggctcgatgatggttacgtaccaggcacagaagggccacccgaattttttccgtattgtgttccaaaatagcggactcgataaagctgatatggtccaccttgtcgaagagatcgaacggcttggttcagatttgtaa